European Patent Specification EP 3 997 216 B1, published April 8, 2026. Title: ENGINEERED ALPHA-1,3 BRANCHING ENZYMES. Applicant: NUTRITION & BIOSCIENCES USA 4, INC. Li, Yougen Semke, Ellen. The sequence listing filed with the application follows.

SEQUENCE LISTING (15 sequences)

SEQ ID NO: 1 - DNA, 5229 bp, Artificial sequence
  encoding GTF 2592, truncated, w/ added start methionine and C-terminal 6xHis tag
atgacaactgtagcaagtgctgatgtacaaaaggatacagtagttgttactgcagataaaaatactactgataaggacaaagaaccgattaagacagcgggagcaaatgttgttgataagggagttgcccagacaacggacacaaatactactgataaaaagacgatagaagtaggtaagtcagtagacatgagtgctactgataagaaagtgacagaaacagttaaatcagtggacacgagtgctactgataaaaagacaacagaagctgttaaaccagtagatacgaatgctactgataagaaagcaacagaagcagttaagccagtagatacgaatgctactgataagaagacgacagaagcagttaagccagtagacacaaatactactgataagaaagtaacagaagcaattaagccagtaaacacaaatgctgatgataagacagcagagcctgttaagacaatatcagcaaccaaagataccgttaaaaccatagctaataagcaaaagggggcaactgaagagcaagcagttattactgaagggcattacgaagcccaaggtgatggttttgtttatattactaaagatggtaaacaattaacgggattacagaatattaatggtaatactcaatactttgatcctgcaacaggacaacagctgaagggcgatattaaagcagttgcaggcacagtctattactttgataaaaatagcggtaatgcacgcgtataccaaaaagtagcagatggtacttattcagagaataatgagcattggcaatatatcagtaaagtagataataagccggttgagggcttatataatgtacaaggtaacctacaatactttgatatgtccactggaaatcaagtaaaaaatgatattcgctctgtggacggcgtcacttactattttgacaaagatagtggtaatggatcagcatttaatgcattatcagctggtgaatacgttgaaaagaaggagacggacgcacaaggcaatcagaactcatattggacatatagtggattagatggtaatccggttaaaggattgtatgatattaacggttcactacaatattttgatgaaaagaatggtgcacagttaaaaggtggaacagccacagtcaatggcgtaacatattattttgaacaagataagggtaacctgattagtgttgttaatagtgttgagagtggtcaatataaaattgataatgacaacgtttattatattgacaatcaaggtaacacgttaaaaggtctatatgctattaatggacaattaaattattttgacatgagcactggtgttcaactaaaaggtgctagtgagaatgctaatggtgtcggttattacttcgataaagataagggtaatggtcagtatcaatatagtttgattacttcgacacttgctaatgcattttcaaaacataatgcagctaatgattacactcagagtagttttactcatactgttgatggctttttgacagctgatacgtggtaccgaccaacagagatactcaaaaatggaacgacatgggttgcttcaacatcacaggatttgagaccaatgattactgtttggtggcctaataaaaatgtacagcttaactatcttaaacttatgcaaacagaagggttgttggatagtggccaagtatatgatttgaatagcgatcaagcactgctcaatcaagcagcacaaacggtgcaagtgaacattgaaaaaaggataactaaagcaggaaattctgattggcttaatgatttgctatataacagtcacggtgaaacaccttcgtttgttaagcagcaggctatttggaatgctgattctgaatatcatggcggttggttccagggtggatatttagcatatcggaatagtgatttaacaccatatgcgaattcatcatacagacattacaccggaatggaatttttgttggctaatgatgttgataattccaatccaattgtacaagctgaagaccttaactggttatactatctaatgaattttggaacggaaacaggcaatgatccgcaagccaattttgatagtatccgtattgatgctattagctttgtcgacaaacaagtggctaagaaagcatatgaattacttcatgatatgtatggcttatcagctagtgacgctgtagcaaataagcatgtttctattgtagaagcaagtgccgatcagacaccagttacgacagaaaatcatgatgcattaattgagtcttactggcgtgacactatgaaaaattcattgtccaaagatgcgtcaattgattcatctgctggatcgttatctgcaatgataaatgatggaaatgttgatcgtgctaacgatagtactacagaaagttcaatattcccaaactatacaattgttcatgcgcatgataaagatatacaagatgctgtaagcaatgttatgaaaattgtaaataatgatccatccatttcactagatggttttacaatggaacagttagagaagggattgtcagcattttatgctgatcagagatctgctgttaagcaatataatcaatataatattccaagtgcttatgcggttatgttaactaacaaagatactgtgccacgtacattttatggtgatatgtatcaagatgatggtcaatatatggctaataagtcactatactatgatgctattgatacaatgatgaaggctcgcctgaaatatgtttccggtggtcaaactatgtctgttacaaaaatcaataatgcaaatagtcagaaatctggagaagtattaacaagcgttcgttttggaaaaggtgttatggatgctacagatgccggaagtgctgaaagtagaacacaaggcattggtgtggttgtgtctaatagtagcggtcttcaattgaacgataatgataaaattgtgttacatatgggtgcggcgcataaaaaccaagaataccgtgcattaatgttaacaactaatgatggtattaaatcctttaataacgatgaagcaccaattaattatactgatgataatggtgatttaatttttgatggacacaatattgatggtcaagagaatacagcaatcagaggttatcttaatccgcaagttgctggatatttagcggtatgggtaccaactggtgctaaagatgatcaagatgctagaacacaaccttccaatgaaaaatctactgatggcaaagtattacacacaaatgctgctttggattctgaattgatttatgaaggattttctaacttccaacccatgccaacaactaaagatgaatatacgaatgtgatgattgctaaaaatattgatctctttaagtcatggggtatcactaattttgaattagcaccacaatatcgatcaagcgatggcaaaaatattaatgatcgttttattgattcacttgttcagaatggttatggtttgagcgaccgatacgatcttgggtttgagacgccaactaaatatggtacagatcaagatttgagaacagcgattaaaacattacaccaagccggtatgactgtcatggctgactatgttgctaaccaaatttatggattgaatacaagtcaagaagtggttgatgcgcaacgagttaattcggataataatgcagtcgaagttcgctacggtcagcatttgaatgttgtaaactcaattgggggcggtgaatatcagaatttgtatggtggaaaatacctagaaattttgaataaactttatcctgatctgctggtcgatgagaatggtaataaaatagatattgataccaaaatcaaacaatggtctgctaaatatcttaacggcagtaatgtaaccggactcggtatggggtatgttctaaaagattggtcaaatggacaatactttaatatttctaatactgatggcaaagttatgttgccagaacagttagttaaacatatgcctgccgtagaaattggtacgcaaacgaattatacggcgtatatttcaagtacaattcgtcgtgatggtctttataacaatatgccatggggtgtcactgctacaggacaagatggcaacgagataaagtgggaacgtcaaggtagtacgtctgattataatcaccagaaggtacaagtaaaccgacagtatgttgataagcaaggtgttgtttggaacttaattaattttgatgataaagatctatgggttgatagtaatgcactcgtaacggttaactttacatcacaaaagccaactaagcattttgtccaattcggtatgcgtcaaggtaagtatgatggcttctatcttagtgcaccatataagcaaactgagtcaaagtgggttgcttctacacgaacacatcaaggacaattattggaagttgtcggtcaatatacaacagggtcaggtagtcgtaaggtaacttggtacttggttggtcttgatggtaagcaagtatgggtagacagtcgagctgttggtactaatttcagtcataagacaaatattaatttgttgattaatagtgccacacgcaatgatggtatgtacttgaatgcaccgtatggtcagaagggttataagcgagaaacatcaagtcgcttctataatgaaaagctcgtaacagttagtcaacaatattacgataataagggtgttatttggaaccttattactttgaatggtaaaaagctgtgggtagatagccgagcatttgcaacagttattgataagaaagtgaaccaaagcctgtatatcaatagtcgtaatgatggtatgtacttgaatgcaccatatcgtgcacaaggtgctaaacgatatgcttcaacgaagacatatacagggcaacgtgtgcaagtgacattacaacgtaaagatactcacggtgtaacttggtatctcactaaggtagatagtaagcagttgtgggtagacagccatgcatttgcaccaaccttcacgcgtaatgtgtcgctcaatgttaaagtgaacagttcaaaacgtaatgatgggatttacttaaacgcaccatatggcaataaaaaagccaagcgtattgcatcaacaaaggcatacaatggtaagcgtgtaaaagctagtaaagaatataaagatgctaagggagtaacttggtatttggtaaaccttaataataaacaagtgtggattgacaaacgtgcatttcaccatcaccaccatcactaa

SEQ ID NO: 2 - protein, 1742 aa, Artificial sequence
  GTF 2592, truncated, w/ added start methionine and C-terminal 6xHis tag
MTTVASADVQKDTVVVTADKNTTDKDKEPIKTAGANVVDKGVAQTTDTNTTDKKTIEVGKSVDMSATDKKVTETVKSVDTSATDKKTTEAVKPVDTNATDKKATEAVKPVDTNATDKKTTEAVKPVDTNTTDKKVTEAIKPVNTNADDKTAEPVKTISATKDTVKTIANKQKGATEEQAVITEGHYEAQGDGFVYITKDGKQLTGLQNINGNTQYFDPATGQQLKGDIKAVAGTVYYFDKNSGNARVYQKVADGTYSENNEHWQYISKVDNKPVEGLYNVQGNLQYFDMSTGNQVKNDIRSVDGVTYYFDKDSGNGSAFNALSAGEYVEKKETDAQGNQNSYWTYSGLDGNPVKGLYDINGSLQYFDEKNGAQLKGGTATVNGVTYYFEQDKGNLISVVNSVESGQYKIDNDNVYYIDNQGNTLKGLYAINGQLNYFDMSTGVQLKGASENANGVGYYFDKDKGNGQYQYSLITSTLANAFSKHNAANDYTQSSFTHTVDGFLTADTWYRPTEILKNGTTWVASTSQDLRPMITVWWPNKNVQLNYLKLMQTEGLLDSGQVYDLNSDQALLNQAAQTVQVNIEKRITKAGNSDWLNDLLYNSHGETPSFVKQQAIWNADSEYHGGWFQGGYLAYRNSDLTPYANSSYRHYTGMEFLLANDVDNSNPIVQAEDLNWLYYLMNFGTETGNDPQANFDSIRIDAISFVDKQVAKKAYELLHDMYGLSASDAVANKHVSIVEASADQTPVTTENHDALIESYWRDTMKNSLSKDASIDSSAGSLSAMINDGNVDRANDSTTESSIFPNYTIVHAHDKDIQDAVSNVMKIVNNDPSISLDGFTMEQLEKGLSAFYADQRSAVKQYNQYNIPSAYAVMLTNKDTVPRTFYGDMYQDDGQYMANKSLYYDAIDTMMKARLKYVSGGQTMSVTKINNANSQKSGEVLTSVRFGKGVMDATDAGSAESRTQGIGVVVSNSSGLQLNDNDKIVLHMGAAHKNQEYRALMLTTNDGIKSFNNDEAPINYTDDNGDLIFDGHNIDGQENTAIRGYLNPQVAGYLAVWVPTGAKDDQDARTQPSNEKSTDGKVLHTNAALDSELIYEGFSNFQPMPTTKDEYTNVMIAKNIDLFKSWGITNFELAPQYRSSDGKNINDRFIDSLVQNGYGLSDRYDLGFETPTKYGTDQDLRTAIKTLHQAGMTVMADYVANQIYGLNTSQEVVDAQRVNSDNNAVEVRYGQHLNVVNSIGGGEYQNLYGGKYLEILNKLYPDLLVDENGNKIDIDTKIKQWSAKYLNGSNVTGLGMGYVLKDWSNGQYFNISNTDGKVMLPEQLVKHMPAVEIGTQTNYTAYISSTIRRDGLYNNMPWGVTATGQDGNEIKWERQGSTSDYNHQKVQVNRQYVDKQGVVWNLINFDDKDLWVDSNALVTVNFTSQKPTKHFVQFGMRQGKYDGFYLSAPYKQTESKWVASTRTHQGQLLEVVGQYTTGSGSRKVTWYLVGLDGKQVWVDSRAVGTNFSHKTNINLLINSATRNDGMYLNAPYGQKGYKRETSSRFYNEKLVTVSQQYYDNKGVIWNLITLNGKKLWVDSRAFATVIDKKVNQSLYINSRNDGMYLNAPYRAQGAKRYASTKTYTGQRVQVTLQRKDTHGVTWYLTKVDSKQLWVDSHAFAPTFTRNVSLNVKVNSSKRNDGIYLNAPYGNKKAKRIASTKAYNGKRVKASKEYKDAKGVTWYLVNLNNKQVWIDKRAFHHHHHH

SEQ ID NO: 3 - protein, 1735 aa, Leuconostoc fallax
TTVASADVQKDTVVVTADKNTTDKDKEPIKTAGANVVDKGVAQTTDTNTTDKKTIEVGKSVDMSATDKKVTETVKSVDTSATDKKTTEAVKPVDTNATDKKATEAVKPVDTNATDKKTTEAVKPVDTNTTDKKVTEAIKPVNTNADDKTAEPVKTISATKDTVKTIANKQKGATEEQAVITEGHYEAQGDGFVYITKDGKQLTGLQNINGNTQYFDPATGQQLKGDIKAVAGTVYYFDKNSGNARVYQKVADGTYSENNEHWQYISKVDNKPVEGLYNVQGNLQYFDMSTGNQVKNDIRSVDGVTYYFDKDSGNGSAFNALSAGEYVEKKETDAQGNQNSYWTYSGLDGNPVKGLYDINGSLQYFDEKNGAQLKGGTATVNGVTYYFEQDKGNLISVVNSVESGQYKIDNDNVYYIDNQGNTLKGLYAINGQLNYFDMSTGVQLKGASENANGVGYYFDKDKGNGQYQYSLITSTLANAFSKHNAANDYTQSSFTHTVDGFLTADTWYRPTEILKNGTTWVASTSQDLRPMITVWWPNKNVQLNYLKLMQTEGLLDSGQVYDLNSDQALLNQAAQTVQVNIEKRITKAGNSDWLNDLLYNSHGETPSFVKQQAIWNADSEYHGGWFQGGYLAYRNSDLTPYANSSYRHYTGMEFLLANDVDNSNPIVQAEDLNWLYYLMNFGTETGNDPQANFDSIRIDAISFVDKQVAKKAYELLHDMYGLSASDAVANKHVSIVEASADQTPVTTENHDALIESYWRDTMKNSLSKDASIDSSAGSLSAMINDGNVDRANDSTTESSIFPNYTIVHAHDKDIQDAVSNVMKIVNNDPSISLDGFTMEQLEKGLSAFYADQRSAVKQYNQYNIPSAYAVMLTNKDTVPRTFYGDMYQDDGQYMANKSLYYDAIDTMMKARLKYVSGGQTMSVTKINNANSQKSGEVLTSVRFGKGVMDATDAGSAESRTQGIGVVVSNSSGLQLNDNDKIVLHMGAAHKNQEYRALMLTTNDGIKSFNNDEAPINYTDDNGDLIFDGHNIDGQENTAIRGYLNPQVAGYLAVWVPTGAKDDQDARTQPSNEKSTDGKVLHTNAALDSELIYEGFSNFQPMPTTKDEYTNVMIAKNIDLFKSWGITNFELAPQYRSSDGKNINDRFIDSLVQNGYGLSDRYDLGFETPTKYGTDQDLRTAIKTLHQAGMTVMADYVANQIYGLNTSQEVVDAQRVNSDNNAVEVRYGQHLNVVNSIGGGEYQNLYGGKYLEILNKLYPDLLVDENGNKIDIDTKIKQWSAKYLNGSNVTGLGMGYVLKDWSNGQYFNISNTDGKVMLPEQLVKHMPAVEIGTQTNYTAYISSTIRRDGLYNNMPWGVTATGQDGNEIKWERQGSTSDYNHQKVQVNRQYVDKQGVVWNLINFDDKDLWVDSNALVTVNFTSQKPTKHFVQFGMRQGKYDGFYLSAPYKQTESKWVASTRTHQGQLLEVVGQYTTGSGSRKVTWYLVGLDGKQVWVDSRAVGTNFSHKTNINLLINSATRNDGMYLNAPYGQKGYKRETSSRFYNEKLVTVSQQYYDNKGVIWNLITLNGKKLWVDSRAFATVIDKKVNQSLYINSRNDGMYLNAPYRAQGAKRYASTKTYTGQRVQVTLQRKDTHGVTWYLTKVDSKQLWVDSHAFAPTFTRNVSLNVKVNSSKRNDGIYLNAPYGNKKAKRIASTKAYNGKRVKASKEYKDAKGVTWYLVNLNNKQVWIDKRAF

SEQ ID NO: 4 - protein, 1774 aa, Leuconostoc fallax
MKQQESITRKKLYKAGKSWVVAATLFAATLFAAMGAAGATTVASADVQKDTVVVTADKNTTDKDKEPIKTAGANVVDKGVAQTTDTNTTDKKTIEVGKSVDMSATDKKVTETVKSVDTSATDKKTTEAVKPVDTNATDKKATEAVKPVDTNATDKKTTEAVKPVDTNTTDKKVTEAIKPVNTNADDKTAEPVKTISATKDTVKTIANKQKGATEEQAVITEGHYEAQGDGFVYITKDGKQLTGLQNINGNTQYFDPATGQQLKGDIKAVAGTVYYFDKNSGNARVYQKVADGTYSENNEHWQYISKVDNKPVEGLYNVQGNLQYFDMSTGNQVKNDIRSVDGVTYYFDKDSGNGSAFNALSAGEYVEKKETDAQGNQNSYWTYSGLDGNPVKGLYDINGSLQYFDEKNGAQLKGGTATVNGVTYYFEQDKGNLISVVNSVESGQYKIDNDNVYYIDNQGNTLKGLYAINGQLNYFDMSTGVQLKGASENANGVGYYFDKDKGNGQYQYSLITSTLANAFSKHNAANDYTQSSFTHTVDGFLTADTWYRPTEILKNGTTWVASTSQDLRPMITVWWPNKNVQLNYLKLMQTEGLLDSGQVYDLNSDQALLNQAAQTVQVNIEKRITKAGNSDWLNDLLYNSHGETPSFVKQQAIWNADSEYHGGWFQGGYLAYRNSDLTPYANSSYRHYTGMEFLLANDVDNSNPIVQAEDLNWLYYLMNFGTETGNDPQANFDSIRIDAISFVDKQVAKKAYELLHDMYGLSASDAVANKHVSIVEASADQTPVTTENHDALIESYWRDTMKNSLSKDASIDSSAGSLSAMINDGNVDRANDSTTESSIFPNYTIVHAHDKDIQDAVSNVMKIVNNDPSISLDGFTMEQLEKGLSAFYADQRSAVKQYNQYNIPSAYAVMLTNKDTVPRTFYGDMYQDDGQYMANKSLYYDAIDTMMKARLKYVSGGQTMSVTKINNANSQKSGEVLTSVRFGKGVMDATDAGSAESRTQGIGVVVSNSSGLQLNDNDKIVLHMGAAHKNQEYRALMLTTNDGIKSFNNDEAPINYTDDNGDLIFDGHNIDGQENTAIRGYLNPQVAGYLAVWVPTGAKDDQDARTQPSNEKSTDGKVLHTNAALDSELIYEGFSNFQPMPTTKDEYTNVMIAKNIDLFKSWGITNFELAPQYRSSDGKNINDRFIDSLVQNGYGLSDRYDLGFETPTKYGTDQDLRTAIKTLHQAGMTVMADYVANQIYGLNTSQEVVDAQRVNSDNNAVEVRYGQHLNVVNSIGGGEYQNLYGGKYLEILNKLYPDLLVDENGNKIDIDTKIKQWSAKYLNGSNVTGLGMGYVLKDWSNGQYFNISNTDGKVMLPEQLVKHMPAVEIGTQTNYTAYISSTIRRDGLYNNMPWGVTATGQDGNEIKWERQGSTSDYNHQKVQVNRQYVDKQGVVWNLINFDDKDLWVDSNALVTVNFTSQKPTKHFVQFGMRQGKYDGFYLSAPYKQTESKWVASTRTHQGQLLEVVGQYTTGSGSRKVTWYLVGLDGKQVWVDSRAVGTNFSHKTNINLLINSATRNDGMYLNAPYGQKGYKRETSSRFYNEKLVTVSQQYYDNKGVIWNLITLNGKKLWVDSRAFATVIDKKVNQSLYINSRNDGMYLNAPYRAQGAKRYASTKTYTGQRVQVTLQRKDTHGVTWYLTKVDSKQLWVDSHAFAPTFTRNVSLNVKVNSSKRNDGIYLNAPYGNKKAKRIASTKAYNGKRVKASKEYKDAKGVTWYLVNLNNKQVWIDKRAF

SEQ ID NO: 5 - protein, 7 aa, Leuconostoc fallax
ADYVANQ

SEQ ID NO: 6 - protein, 11 aa, Leuconostoc fallax
SIRIDAISFVD

SEQ ID NO: 7 - protein, 11 aa, Leuconostoc fallax
HVSIVEASADQ

SEQ ID NO: 8 - protein, 15 aa, Leuconostoc fallax
IVHAHDKDIQDAVSN

SEQ ID NO: 9 - protein, 7 aa, Unknown
  Alpha-1,3-branching enzyme conserved motif I
  MISC_FEATURE (3)..(3): Xaa is Phe or Tyr
ADXVANQ

SEQ ID NO: 10 - protein, 11 aa, Unknown
  Alpha-1,3-branching enzyme conserved motif II
  MISC_FEATURE (2)..(2): Xaa is Met or Ile
SXRIDAISFVD

SEQ ID NO: 11 - protein, 11 aa, Unknown
  Alpha-1,3-branching enzyme conserved motif III
  MISC_FEATURE (2)..(2): Xaa is Val or Ile
  MISC_FEATURE (8)..(8): Xaa is Pro or Ser
  MISC_FEATURE (9)..(9): Xaa is Lys or Ala
  MISC_FEATURE (10)..(10): Xaa is Gly or Asp
  MISC_FEATURE (11)..(11): Xaa is Glu or Gln
HXSIVEAXXXX

SEQ ID NO: 12 - protein, 15 aa, Unknown
  Alpha-1,3-branching enzyme conserved motif IV
  MISC_FEATURE (12)..(12): Xaa is Thr or Ala
  MISC_FEATURE (14)..(14): Xaa is Ser or Ile
  MISC_FEATURE (15)..(15): Xaa is His or Asn
IVHAHDKDIQDXVXX

SEQ ID NO: 13 - protein, 1888 aa, Leuconostoc citreum
MEMKETITRKKLYKSGKSWVAAATAFAVMGVSAVTTVSADTQTPVGTTQSQQDLTGQTGQDKPTTKEVIDKKEPVPQVSAQNVGDLSADAKTPKADDKQDTQPTNAQLPDQGNKQTNSNSDKGVKESTTAPVKTTDVPSKSVAPETNTSINGGQYVEKDGQFVYIDQSGKQVSGLQNIEGHTQYFDPKTGYQTKGELKNIDDNAYYFDKNSGNGRTFTKISNGSYSEKDGMWQYVDSHDKQPVKGLYDVEGNLQYFDLSTGNQAKHQIRSVDGVTYYFDADSGNATAFKAVTNGRYAEQTTKDKDGNETSYWAYLDNQGNAIKGLNDVNGEIQYFDEHTGEQLKGHTATVDGTTYYFEGNKGNLVSVVNTAPTGQYKINGDNVYYLDNNNEAIKGLYGINGNLNYFDLATGIQLKGQAKNIDGIGYYFDQNNGNGEYRYSLTGPVVKDVYSQHNAVNNLSANNFKNLVDGFLTAETWYRPAQILSHGTDWVASTDKDFRPLITVWWPNKDIQVNYLKLMQQIGILDNSVVFDTNNDQLVLNKGAESAQIGIEKKVSETGNTDWLNELLFAPNGNQPSFIKQQYLWNVDSEYPGGWFQGGYLAYQNSDLTPYANTNPDYRTHNGLEFLLANDVDNSNPVVQAEQLNWLYYLMNFGQITANDSNANFDSMRIDAISFVDPQIAKKAYDLLDKMYGLTDNEAVANQHISIVEAPKGETPITVEKQSALVESNWRDRMKQSLSKNATLDKLDPDPAINSLEKLVADDLVNRSQSSDKDSSTIPNYSIVHAHDKDIQDTVIHIMKIVNNNPNISMSDFTMQQLQNGLKAFYEDQHQSVKKYNQYNIPSAYALLLTNKDTVPRVFYGDMYQDYGDDLDGGQYMATKSIYYNAIEQMMKARLKYVAGGQIMAVTKIKNDGINKDGTNKSGEVLTSVRFGKDIMDAQGQGTAESRNQGIGVIVSNSSGLELKNSDSITLHMGIAHKNQAYRALMLTNDKGIVNYDQDNNAPIAWTNDHGDLIFTNQMINGQSDTAVKGYLNPEVAGYLAVWVPVGANDNQDARTVTTNQKNTDGKVLHTNAALDSKLMYEGFSNFQKMPTRGNQYANVVITKNIDLFKSWGITDFELAPQYRSSDGKDITDRFLDSIVQNGYGLSDRYDLGFKTPTKYGTDQDLRKAIERLHQAGMSVMADFVANQIYGLHADKEVVSAQHVNINGDTKLVVDPRYGTQMTVVNSVGGGDYQAKYGGEYLDTISKLYPGLLLDSNGQKIDLSTKIKEWSAKYLNGSNIPQVGMGYVLKDWNNGQYFHILDKEGQYSLPTQLVSNDPETQIGESVNYKYFIGNSDATYNMYHNLPNTVSLINSQEGQIKTQQSGVTSDYEGQQVQVTRQYTDSKGVSWNLITFAGGDLQGQKLWVDSRALTMTPFKTMNQISFISYANRNDGLFLNAPYQVKGYQLAGMSNQYKGQQVTIAGVANVSGKDWSLISFNGTQYWIDSQALNTNFTHDMNQKVFVNTTSNLDGLFLNAPYRQPGYKLAGLAKNYNNQTVTVSQQYFDDQGTVWSEVVLGGQTVWVDNHALAQMQVSDTSQQLYVNSNGRNDGLFLNAPYRGQGSQLIGMTADYNGQHVQVTKQGQDAYGAQWRLITLNNQQVWVDSRALSTTIVQAMNDDMYVNSNQRTDGLWLNAPYTMSGAKWAGDTRSANGRYVHISKAYSNEVGNTYYLTNLNGQSTWIDKRAFTATFDQVVALNATIVARQRPDGMFKTAPYGEAGAQFVDYVTNYNQQTVPVTKQHSDAQGNQWYLATVNGTQYWIDQRSFSPVVTKVVDYQAKIVPRTTRDGVFSGAPYGEVNAKLVNMATAYQNQVVHATGEYTNASGITWSQFALSGQEDKLWIDKRALQA

SEQ ID NO: 14 - protein, 868 aa, Leuconostoc citreum
VKDVYSQHNAVNNLSANNFKNLVDGFLTAETWYRPAQILSHGTDWVASTDKDFRPLITVWWPNKDIQVNYLKLMQQIGILDNSVVFDTNNDQLVLNKGAESAQIGIEKKVSETGNTDWLNELLFAPNGNQPSFIKQQYLWNVDSEYPGGWFQGGYLAYQNSDLTPYANTNPDYRTHNGLEFLLANDVDNSNPVVQAEQLNWLYYLMNFGQITANDSNANFDSMRIDAISFVDPQIAKKAYDLLDKMYGLTDNEAVANQHISIVEAPKGETPITVEKQSALVESNWRDRMKQSLSKNATLDKLDPDPAINSLEKLVADDLVNRSQSSDKDSSTIPNYSIVHAHDKDIQDTVIHIMKIVNNNPNISMSDFTMQQLQNGLKAFYEDQHQSVKKYNQYNIPSAYALLLTNKDTVPRVFYGDMYQDYGDDLDGGQYMATKSIYYNAIEQMMKARLKYVAGGQIMAVTKIKNDGINKDGTNKSGEVLTSVRFGKDIMDAQGQGTAESRNQGIGVIVSNSSGLELKNSDSITLHMGIAHKNQAYRALMLTNDKGIVNYDQDNNAPIAWTNDHGDLIFTNQMINGQSDTAVKGYLNPEVAGYLAVWVPVGANDNQDARTVTTNQKNTDGKVLHTNAALDSKLMYEGFSNFQKMPTRGNQYANVVITKNIDLFKSWGITDFELAPQYRSSDGKDITDRFLDSIVQNGYGLSDRYDLGFKTPTKYGTDQDLRKAIERLHQAGMSVMADFVANQIYGLHADKEVVSAQHVNINGDTKLVVDPRYGTQMTVVNSVGGGDYQAKYGGEYLDTISKLYPGLLLDSNGQKIDLSTKIKEWSAKYLNGSNIPQVGMGYVLKDWNNGQYFHILDKEGQYSLPTQL

SEQ ID NO: 15 - protein, 1849 aa, Leuconostoc citreum
DTQTPVGTTQSQQDLTGQTGQDKPTTKEVIDKKEPVPQVSAQNVGDLSADAKTPKADDKQDTQPTNAQLPDQGNKQTNSNSDKGVKESTTAPVKTTDVPSKSVAPETNTSINGGQYVEKDGQFVYIDQSGKQVSGLQNIEGHTQYFDPKTGYQTKGELKNIDDNAYYFDKNSGNGRTFTKISNGSYSEKDGMWQYVDSHDKQPVKGLYDVEGNLQYFDLSTGNQAKHQIRSVDGVTYYFDADSGNATAFKAVTNGRYAEQTTKDKDGNETSYWAYLDNQGNAIKGLNDVNGEIQYFDEHTGEQLKGHTATVDGTTYYFEGNKGNLVSVVNTAPTGQYKINGDNVYYLDNNNEAIKGLYGINGNLNYFDLATGIQLKGQAKNIDGIGYYFDQNNGNGEYRYSLTGPVVKDVYSQHNAVNNLSANNFKNLVDGFLTAETWYRPAQILSHGTDWVASTDKDFRPLITVWWPNKDIQVNYLKLMQQIGILDNSVVFDTNNDQLVLNKGAESAQIGIEKKVSETGNTDWLNELLFAPNGNQPSFIKQQYLWNVDSEYPGGWFQGGYLAYQNSDLTPYANTNPDYRTHNGLEFLLANDVDNSNPVVQAEQLNWLYYLMNFGQITANDSNANFDSMRIDAISFVDPQIAKKAYDLLDKMYGLTDNEAVANQHISIVEAPKGETPITVEKQSALVESNWRDRMKQSLSKNATLDKLDPDPAINSLEKLVADDLVNRSQSSDKDSSTIPNYSIVHAHDKDIQDTVIHIMKIVNNNPNISMSDFTMQQLQNGLKAFYEDQHQSVKKYNQYNIPSAYALLLTNKDTVPRVFYGDMYQDYGDDLDGGQYMATKSIYYNAIEQMMKARLKYVAGGQIMAVTKIKNDGINKDGTNKSGEVLTSVRFGKDIMDAQGQGTAESRNQGIGVIVSNSSGLELKNSDSITLHMGIAHKNQAYRALMLTNDKGIVNYDQDNNAPIAWTNDHGDLIFTNQMINGQSDTAVKGYLNPEVAGYLAVWVPVGANDNQDARTVTTNQKNTDGKVLHTNAALDSKLMYEGFSNFQKMPTRGNQYANVVITKNIDLFKSWGITDFELAPQYRSSDGKDITDRFLDSIVQNGYGLSDRYDLGFKTPTKYGTDQDLRKAIERLHQAGMSVMADFVANQIYGLHADKEVVSAQHVNINGDTKLVVDPRYGTQMTVVNSVGGGDYQAKYGGEYLDTISKLYPGLLLDSNGQKIDLSTKIKEWSAKYLNGSNIPQVGMGYVLKDWNNGQYFHILDKEGQYSLPTQLVSNDPETQIGESVNYKYFIGNSDATYNMYHNLPNTVSLINSQEGQIKTQQSGVTSDYEGQQVQVTRQYTDSKGVSWNLITFAGGDLQGQKLWVDSRALTMTPFKTMNQISFISYANRNDGLFLNAPYQVKGYQLAGMSNQYKGQQVTIAGVANVSGKDWSLISFNGTQYWIDSQALNTNFTHDMNQKVFVNTTSNLDGLFLNAPYRQPGYKLAGLAKNYNNQTVTVSQQYFDDQGTVWSEVVLGGQTVWVDNHALAQMQVSDTSQQLYVNSNGRNDGLFLNAPYRGQGSQLIGMTADYNGQHVQVTKQGQDAYGAQWRLITLNNQQVWVDSRALSTTIVQAMNDDMYVNSNQRTDGLWLNAPYTMSGAKWAGDTRSANGRYVHISKAYSNEVGNTYYLTNLNGQSTWIDKRAFTATFDQVVALNATIVARQRPDGMFKTAPYGEAGAQFVDYVTNYNQQTVPVTKQHSDAQGNQWYLATVNGTQYWIDQRSFSPVVTKVVDYQAKIVPRTTRDGVFSGAPYGEVNAKLVNMATAYQNQVVHATGEYTNASGITWSQFALSGQEDKLWIDKRALQA